European Patent Specification EP 3 634 998 B1, published February 26, 2025. Title: NOVEL ANTI-CD3 ANTIBODIES. Applicant: Numab Innovation AG. The sequence listing filed with the application follows.

SEQUENCE LISTING (42 sequences)

SEQ ID NO: 1 - protein, 13 aa, Artificial Sequence
  artificial CDR sequence
QSSQSVFSNNYLA

SEQ ID NO: 2 - protein, 7 aa, Artificial Sequence
  artificial CDR sequence
SASTLAS

SEQ ID NO: 3 - protein, 13 aa, Artificial Sequence
  artificial CDR sequence
LGSYACSSADCYV

SEQ ID NO: 4 - protein, 114 aa, Artificial Sequence
  artificial VL sequence
DIQMTQSPSSLSASVGDRVTITCQSSQSVFSNNYLAWFQQKPGQSPKRLIYSASTLASGVPSRFSGSGSGTDFTLTISSLQPEDFATYYCLGSYACSSADCYVFGTGTKVTVLG

SEQ ID NO: 5 - protein, 10 aa, Artificial Sequence
  artificial CDR sequence
GFSLSSYDMS

SEQ ID NO: 6 - protein, 16 aa, Artificial Sequence
  artificial CDR sequence
ASYASGPTYYASWAKG

SEQ ID NO: 7 - protein, 12 aa, Artificial Sequence
  artificial CDR sequence
RGGWTGTSHSNI

SEQ ID NO: 8 - protein, 119 aa, Artificial Sequence
  artificial VH sequence
EVQLVESGGGLVQPGGSLRLSCAASGFSLSSYDMSWVRQAPGKGLAWIGASYASGPTYYASWAKGRFTISRDNSKNTVYLQMNSLRAEDTATYFCARGGWTGTSHSNIWGQGTLVTVSS

SEQ ID NO: 9 - protein, 114 aa, Artificial Sequence
  artificial VL sequence
DIQMTQSPSSLSASVGDRVTITCQSSESVYNNKRLSWYQQKPGKAPKLLIYTASSLASGVPSRFSGSGSGTDFTLTISSLQPEDFATYYCQGEFTCSNADCFTFGTGTKVTVLG

SEQ ID NO: 10 - protein, 123 aa, Artificial Sequence
  artificial VH sequence
EVQLVESGGGLVQPGGSLRLSCAASGFPLSSYAMIWVRQAPGKGLEWIGMILRAGNIYYASWVKGRFTISRDNSKNTVYLQMNSLRAEDTAVYYCARRHYNREGYPIGIGDLWGQGTLVTVSS

SEQ ID NO: 11 - protein, 113 aa, Artificial Sequence
  artificial VL sequence
DIQMTQSPSSLSASVGDRVTITCQASENIYSFLAWYQQKPGKAPKLLIYSASKLAAGVPSRFSGSGSGTDFTLTISSLQPEDFATYYCQQTNRYSNPDIYNVFGTGTKVTVLG

SEQ ID NO: 12 - protein, 121 aa, Artificial Sequence
  artificial VH sequence
EVQLVESGGGLVQPGGSLRLSCAASGIDFNSNYYMCWVRQAPGKGLEWIGCIYVGSHVNTYYANWAKGRFTISRDNSKNTVYLQMNSLRAEDTAVYYCATSGSSVLYFKFWGQGTLVTVSS

SEQ ID NO: 13 - protein, 109 aa, Artificial Sequence
  artificial VL sequence
QTVVTQEPSLTVSPGGTVTLTCGSSTGAVTSGNYPNWVQQKPGQAPRGLIGGTKFLAPGTPARFSGSLLGGKAALTLSGVQPEDEAEYYCVLWYSNRWVFGGGTKLTVL

SEQ ID NO: 14 - protein, 125 aa, Artificial Sequence
  artificial VH sequence
EVQLVESGGGLVQPGGSLKLSCAASGFTFNKYAMNWVRQAPGKGLEWVARIRSKYNNYATYYADSVKDRFTISRDDSKNTAYLQMNNLKTEDTAVYYCVRHGNFGNSYISYWAYWGQGTLVTVSS

SEQ ID NO: 15 - protein, 20 aa, Artificial Sequence
  artificial linker sequence
GGGGSGGGGSGGGGSGGGGS

SEQ ID NO: 16 - protein, 5 aa, Artificial Sequence
  artificial linker sequence
GGGGS

SEQ ID NO: 17 - protein, 11 aa, Artificial Sequence
  artificial FW4 sequence
FGTGTKVTVLG

SEQ ID NO: 18 - protein, 11 aa, Artificial Sequence
  artificial FW4 sequence
FGGGTKLTVLG

SEQ ID NO: 19 - protein, 207 aa, Homo sapiens
MQSGTHWRVLGLCLLSVGVWGQDGNEEMGGITQTPYKVSISGTTVILTCPQYPGSEILWQHNDKNIGGDEDDKNIGSDEDHLSLKEFSELEQSGYYVCYPRGSKPEDANFYLYLRARVCENCMEMDVMSVATIVIVDICITGGLLLLVYYWSKNRKAKAKPVTRGAGAGGRQRGQNKERPPPVPNPDYEPIRKGQRDLYSGLNQRRI

SEQ ID NO: 20 - protein, 108 aa, Artificial Sequence
  artificial VL sequence
DIQMTQSPSSLSASVGDRVTITCRASQDVNTAVAWYQQKPGKAPKLLIYSASFLYSGVPSRFSGSRSGTDFTLTISSLQPEDFATYYCQQHYTTPPTFGTGTKVTVLG

SEQ ID NO: 21 - protein, 120 aa, Artificial Sequence [sequence omitted]

SEQ ID NO: 22 - protein, 112 aa, Artificial Sequence
  artificial VL sequence
DIQMTQSPSSLSASVGDRVTITCQSSESVYSNNQLSWYQQKPGQPPKLLIYDASDLASGVPSRFSGSGSGTDFTLTISSLQPEDFATYYCAGGFSSSSDTAFGGGTKLTVLG

SEQ ID NO: 23 - protein, 121 aa, Artificial Sequence
  artificial VH sequence
EVQLVESGGGLVQPGGSLRLSCAASGFSLSSNAMGWVRQAPGKGLEYIGIISVGGFTYYASWAKGRFTISRDNSKNTVYLQMNSLRAEDTATYFCARDRHGGDSSGAFYLWGQGTLVTVSS

SEQ ID NO: 24 - protein, 110 aa, Artificial Sequence
  artificial VL sequence
DVVMTQSPSSLSASVGDRVTITCQASQIISSRSAWYQQKPGQPPKLLIYQASKLASGVPSRFSGSGSGTDFTLTISSLQPEDFATYYCQCTYIDSNFGAFGGGTKLTVLG

SEQ ID NO: 25 - protein, 121 aa, Artificial Sequence
  artificial VH sequence
EVQLVESGGGLVQPGGSLRLSCAASGFSFSSSYWICWVRQAPGKGLEWVGCVFTGDGTTYYASWAKGRFTISRDNSKNTVYLQMNSLRAEDTATYFCARPVSVYYYGMDLWGQGTLVTVSS

SEQ ID NO: 26 - protein, 497 aa, Artificial Sequence
  artificial diabody sequence
DIQMTQSPSSLSASVGDRVTITCQASENIYSFLAWYQQKPGKAPKLLIYSASKLAAGVPSRFSGSGSGTDFTLTISSLQPEDFATYYCQQTNRYSNPDIYNVFGTGTKVTVLGGGGGSEVQLVESGGGLVQPGGSLRLSCAASGFSLSSYDMSWVRQAPGKGLAWIGASYASGPTYYASWAKGRFTISRDNSKNTVYLQMNSLRAEDTATYFCARGGWTGTSHSNIWGQGTLVTVSSGGGGSGGGGSGGGGSGGGGSDIQMTQSPSSLSASVGDRVTITCQSSQSVFSNNYLAWFQQKPGQSPKRLIYSASTLASGVPSRFSGSGSGTDFTLTISSLQPEDFATYYCLGSYACSSADCYVFGTGTKVTVLGGGGGSEVQLVESGGGLVQPGGSLRLSCAASGIDFNSNYYMCWVRQAPGKGLEWIGCIYVGSHVNTYYANWAKGRFTISRDNSKNTVYLQMNSLRAEDTAVYYCATSGSSVLYFKFWGQGTLVTVSS

SEQ ID NO: 27 - protein, 491 aa, Artificial Sequence
  artificial diabody sequence
DIQMTQSPSSLSASVGDRVTITCRASQDVNTAVAWYQQKPGKAPKLLIYSASFLYSGVPSRFSGSRSGTDFTLTISSLQPEDFATYYCQQHYTTPPTFGTGTKVTVLGGGGGSEVQLVESGGGLVQPGGSLRLSCAASGFSLSSYDMSWVRQAPGKGLAWIGASYASGPTYYASWAKGRFTISRDNSKNTVYLQMNSLRAEDTATYFCARGGWTGTSHSNIWGQGTLVTVSSGGGGSGGGGSGGGGSGGGGSDIQMTQSPSSLSASVGDRVTITCQSSQSVFSNNYLAWFQQKPGQSPKRLIYSASTLASGVPSRFSGSGSGTDFTLTISSLQPEDFATYYCLGSYACSSADCYVFGTGTKVTVLGGGGGSEVQLVESGGGLVQPGGSLRLSCAASGFNIKDTYIHWVRQAPGKGLEWVARIYPTNGYTRYADSVKGRFTISADTSKNTAYLQMNSLRAEDTAVYYCSRWGGDGFYAMDYWGQGTLVTVSS

SEQ ID NO: 28 - protein, 253 aa, Artificial Sequence
  artificial scFv sequence
DIQMTQSPSSLSASVGDRVTITCQSSQSVFSNNYLAWYQQKPGQSPKLLIYSASTLASGVPSRFSGSGSGTDFTLTISSLQPEDFATYYCLGSYACSSADCYVFGTGTKVTVLGGGGGSGGGGSGGGGSGGGGSEVQLVESGGGLVQPGGSLRLSCAASGFSLSSYDMSWVRQAPGKGLEWIGASYASGPTYYASWAKGRFTISRDNSKNTVYLQMNSLRAEDTATYFCARGGWTGTSHSNIWGQGTLVTVSS

SEQ ID NO: 29 - protein, 253 aa, Artificial Sequence
  artificial scFv sequence
DIQMTQSPSSLSASVGDRVTITCQSSQSVFSNNYLAWYQQKPGQSPKRLIYSASTLASGVPSRFSGSGSGTHFTLTISSLQPEDFATYYCLGSYACSSADCYVFGTGTKVTVLGGGGGSGGGGSGGGGSGGGGSEVQLVESGGGLVQPGGSLRLSCAASGFSLSSYDMSWVRQAPGKGLEWIGASYASGPTYYASWAKGRFTISRDNSKNTVYLQMNSLRAEDTATYFCARGGWTGTSHSNIWGQGTLVTVSS

SEQ ID NO: 30 - protein, 253 aa, Artificial Sequence
  artificial scFv sequence
DIQMTQSPSSLSASVGDRVTITCQSSQSVFSNNYLAWYQQKPGQSPKRLIYSASTLASGVPSRFSGSGSGTDFTLTISSLQPEDFATYYCLGSYACSSADCYVFGTGTKVTVLGGGGGSGGGGSGGGGSGGGGSEVQLVESGGGLVQPGGSLRLSCAASGFSLSSYDMSWVRQAPGKGLEWIGASYASGPTYYASWAKGRFTISRDNSKNTVYLQMNSLRAEDTATYFCARGGWTGTSHSNIWGQGTLVTVSS

SEQ ID NO: 31 - protein, 253 aa, Artificial Sequence
  artificial scFv sequence
DIQMTQSPSSLSASVGDRVTITCQSSQSVFSNNYLAWYQQKPGQSPKLLIYSASTLASGVPSRFSGSGSGTHFTLTISSLQPEDFATYYCLGSYACSSADCYVFGTGTKVTVLGGGGGSGGGGSGGGGSGGGGSEVQLVESGGGLVQPGGSLRLSCAASGFSLSSYDMSWVRQAPGKGLEWIGASYASGPTYYASWAKGRFTISRDNSKNTVYLQMNSLRAEDTATYFCARGGWTGTSHSNIWGQGTLVTVSS

SEQ ID NO: 32 - protein, 253 aa, Artificial Sequence
  artificial scFv sequence
DIQMTQSPSSLSASVGDRVTITCQSSQSVFSNNYLAWYQQKPGQSPKRLIYSASTLASGVPSRFSGSGSGTHFTLTISSLQPEDFATYYCLGSYACSSADCYVFGTGTKVTVLGGGGGSGGGGSGGGGSGGGGSEVQLVESGGGLVQPGGSLRLSCAASGFSLSSYDMSWVRQAPGKGLEWIGASYASGPTYYASWAKGRFTISRDNSKNTVYLQMNSLRAEDTAVYYCARGGWTGTSHSNIWGQGTLVTVSS

SEQ ID NO: 33 - protein, 253 aa, Artificial Sequence
  artificial scFv sequence
DIQMTQSPSSLSASVGDRVTITCQSSQSVFSNNYLAWYQQKPGQSPKRLIYSASTLASGVPSRFSGSGSGTDFTLTISSLQPEDFATYYCLGSYACSSADCYVFGTGTKVTVLGGGGGSGGGGSGGGGSGGGGSEVQLVESGGGLVQPGGSLRLSCAASGFSLSSYDMSWVRQAPGKGLEWIGASYASGPTYYASWAKGRFTISRDNSKNTVYLQMNSLRAEDTAVYYCARGGWTGTSHSNIWGQGTLVTVSS

SEQ ID NO: 34 - protein, 253 aa, Artificial Sequence
  artificial scFv sequence
DIQMTQSPSSLSASVGDRVTITCQSSQSVFSNNYLAWYQQKPGQSPKLLIYSASTLASGVPSRFSGSGSGTHFTLTISSLQPEDFATYYCLGSYACSSADCYVFGTGTKVTVLGGGGGSGGGGSGGGGSGGGGSEVQLVESGGGLVQPGGSLRLSCAASGFSLSSYDMSWVRQAPGKGLEWIGASYASGPTYYASWAKGRFTISRDNSKNTVYLQMNSLRAEDTAVYYCARGGWTGTSHSNIWGQGTLVTVSS

SEQ ID NO: 35 - protein, 253 aa, Artificial Sequence
  artificial scFv sequence
DIQMTQSPSSLSASVGDRVTITCQSSQSVFSNNYLAWYQQKPGQSPKRLIYSASTLASGVPSRFSGSGSGTDFTLTISSLQPEDFATYYCLGSYACSSADCYVFGTGTKVTVLGGGGGSGGGGSGGGGSGGGGSEVQLVESGGGLVQPGGSLRLSCAASGFSLSSYDMSWVRQAPGKGLAWIGASYASGPTYYASWAKGRFTISRDNSKNTVYLQMNSLRAEDTAVYYCARGGWTGTSHSNIWGQGTLVTVSS

SEQ ID NO: 36 - protein, 253 aa, Artificial Sequence
  artificial scFv sequence
DIQMTQSPSSLSASVGDRVTITCQSSQSVFSNNYLAWFQQKPGQSPKRLIYSASTLASGVPSRFSGSGSGTDFTLTISSLQPEDFATYYCLGSYACSSADCYVFGTGTKVTVLGGGGGSGGGGSGGGGSGGGGSEVQLVESGGGLVQPGGSLRLSCAASGFSLSSYDMSWVRQAPGKGLEWIGASYASGPTYYASWAKGRFTISRDNSKNTVYLQMNSLRAEDTAVYYCARGGWTGTSHSNIWGQGTLVTVSS

SEQ ID NO: 37 - protein, 253 aa, Artificial Sequence
  artificial scFv sequence
DIQMTQSPSSLSASVGDRVTITCQSSQSVFSNNYLAWYQQKPGKAPKRLIYSASTLASGVPSRFSGSGSGTDFTLTISSLQPEDFATYYCLGSYACSSADCYVFGTGTKVTVLGGGGGSGGGGSGGGGSGGGGSEVQLVESGGGLVQPGGSLRLSCAASGFSLSSYDMSWVRQAPGKGLAWIGASYASGPTYYASWAKGRFTISRDNSKNTVYLQMNSLRAEDTAVYYCARGGWTGTSHSNIWGQGTLVTVSS

SEQ ID NO: 38 - protein, 253 aa, Artificial Sequence
  artificial scFv sequence
DIQMTQSPSSLSASVGDRVTITCQSSQSVFSNNYLAWYQQKPGQSPKKLIYSASTLASGVPSRFSGSGSGTDFTLTISSLQPEDFATYYCLGSYACSSADCYVFGTGTKVTVLGGGGGSGGGGSGGGGSGGGGSEVQLVESGGGLVQPGGSLRLSCAASGFSLSSYDMSWVRQAPGKGLAWIGASYASGPTYYASWAKGRFTISRDNSKNTVYLQMNSLRAEDTAVYYCARGGWTGTSHSNIWGQGTLVTVSS

SEQ ID NO: 39 - protein, 253 aa, Artificial Sequence
  artificial scFv sequence
DIQMTQSPSSLSASVGDRVTITCQSSQSVFSNNYLAWYQQKPGQSPKRLIYSASTLASGVPSRFSGSGSGTDFTLTISSLQPEDFATYYCLGSYACSSADCYVFGTGTKVTVLGGGGGSGGGGSGGGGSGGGGSEVQLVESGGGLVQPGGSLRLSCAASGFSLSSYDMSWVRQAPGKGLAWIGASYASGPTYYASWAKGRFTISRDNSKNTVYLQMNSLRAEDTATYFCARGGWTGTSHSNIWGQGTLVTVSS

SEQ ID NO: 40 - protein, 253 aa, Artificial Sequence
  artificial scFv sequence
DIQMTQSPSSLSASVGDRVTITCQSSQSVFSNNYLAWYQQKPGQSPKRLIYSASTLASGVPSRFSGSGSGTQFTLTISSLQPEDFATYYCLGSYACSSADCYVFGTGTKVTVLGGGGGSGGGGSGGGGSGGGGSEVQLVESGGGLVQPGGSLRLSCAASGFSLSSYDMSWVRQAPGKGLAWIGASYASGPTYYASWAKGRFTISRDNSKNTVYLQMNSLRAEDTAVYYCARGGWTGTSHSNIWGQGTLVTVSS

SEQ ID NO: 41 - protein, 253 aa, Artificial Sequence
  artificial scFv sequence
DIQMTQSPSSLSASVGDRVTITCQSSQSVFSNNYLAWYQQKPGQSPKRLIYSASTLASGVPSRFSGSGSGTDFTLTISSLQPEDFATYYCLGSYACSSADCYVFGTGTKVTVLGGGGGSGGGGSGGGGSGGGGSEVQLVESGGGLVQPGGSLRLSCAVSGFSLSSYDMSWVRQAPGKGLAWIGASYASGPTYYASWAKGRFTISRDNSKNTVYLQMNSLRAEDTAVYYCARGGWTGTSHSNIWGQGTLVTVSS

SEQ ID NO: 42 - protein, 253 aa, Artificial Sequence
  artificial scFv sequence
DIQMTQSPSSLSASVGDRVTITCQSSQSVFSNNYLAWFQQKPGKAPKRLIYSASTLASGVPSRFSGSGSGTDFTLTISSLQPEDFATYYCLGSYACSSADCYVFGTGTKVTVLGGGGGSGGGGSGGGGSGGGGSEVQLVESGGGLVQPGGSLRLSCAASGFSLSSYDMSWVRQAPGKGLEWIGASYASGPTYYASWAKGRFTISRDNSKNTVYLQMNSLRAEDTAVYYCARGGWTGTSHSNIWGQGTLVTVSS